European Patent Application EP 4 177 265 A1, published May 10, 2023. Title: IgA antibodies and kits capable of specifically recognizing RBD protein. Applicant: SHENZHEN YHLO BIOTECH CO., LTD. The sequence listing filed with the application follows.

SEQUENCE LISTING (20 sequences)

SEQ ID NO: 1 - protein, 24 aa, artificial sequence
GGCTACGGCTTCATCACATACTGG

SEQ ID NO: 2 - protein, 24 aa, artificial sequence
ATCTACCCCGGCGACAGCGAGACC

SEQ ID NO: 3 - protein, 36 aa, artificial sequence
GCCGGCGGCTCCGGCATCAGCACCCCTATGGATGTG

SEQ ID NO: 4 - protein, 36 aa, artificial sequence
CAGTCCGTGCTGTACAGCTCCATCAATAAGAATTAC

SEQ ID NO: 5 - protein, 9 aa, artificial sequence
TGGGCCAGC

SEQ ID NO: 6 - protein, 27 aa, artificial sequence
CAGCAGTACTACTCCACACCCTACACA

SEQ ID NO: 7 - protein, 132 aa, artificial sequence
ATGGCCCCAGCCCAGTTTCTGGGCCTGCTGCTGCTGTGTTTCCAGGGCACAAGGTGCCAGATGCAGCTGGTGCAGTCCGGCACAGAGGTGAAGAAGCCTGGCGAGAGCCTGAAGATCAGCTGTAAGGGCTCC

SEQ ID NO: 8 - protein, 51 aa, artificial sequence
ATCGGCTGGGTGAGGCAGATGCCCGGCAAGGGCCTGGAGTGGATGGGCATC

SEQ ID NO: 9 - protein, 114 aa, artificial sequence
AGGTACAGCCCTAGCTTTCAGGGCCAGGTGACCATCAGCGCCGACAAGAGCATCAACACAGCCTACCTGCAGTGGAGCAGCCTGAAGGCCTCCGACACAGCCATCTACTACTGC

SEQ ID NO: 10 - protein, 27 aa, artificial sequence
TGGGGCCAGGGCACAACAGTGACCGTG

SEQ ID NO: 11 - protein, 135 aa, artificial sequence
ATGGCCCCAGCCCAGTTCCTGGGCCTGCTGCTGCTGTGCTTTCAGGGCACAAGATGCGATATCCAGCTGACCCAGTCCCCCGACTCCCTGGCCGTGTCCCTGGGAGAGAGAGCCACAATCAACTGTAAGAGCTCC

SEQ ID NO: 12 - protein, 51 aa, artificial sequence
CTGGCCTGGTACCAGCAGAAGCCTGGCCAGCCTCCCAAGCTGCTGATCTAC

SEQ ID NO: 13 - protein, 108 aa, artificial sequence
ACCAGAGAGTCCGGCGTGCCCGATAGGTTCAGCGGCAGCGGCAGCGGAACAGATTTCACCCTGACCATCAGCAGCCTGCAGGCCGAGGATGTGGCCGTGTACTACTGC

SEQ ID NO: 14 - protein, 30 aa, artificial sequence
TTCGGCCAGGGCACCAAGGTGGAGATCAAG

SEQ ID NO: 15 - protein, 201 aa, artificial sequence
NITNLCPFGEVFNATRFASVYAWNRKRISNCVADYSVLYNSASFSTFKCYGVSPTKLNDLCFTNVYADSFVIRGDEVRQIAPGQTGKIADYNYKLPDDFTGCVIAWNSNNLDSKVGGNYNYLYRLFRKSNLKPFERDISTEIYQAGSTPCNGVEGFNCYFPLQSYGFQPTNGVGYQPYRVVVLSFELLHAPATVCGPKKST

SEQ ID NO: 16 - protein, 23 aa, artificial sequence
ELWLVLVAVGAGLLLLGLIILLL

SEQ ID NO: 17 - protein, 16 aa, artificial sequence
WGQGGTHGQWNKPSKP

SEQ ID NO: 18 - protein, 16 aa, artificial sequence
MFVFLVLLPLVSSQCV

SEQ ID NO: 19 - protein, 1074 aa, Homo sapiens
AGCTCCGCTAGCGCATCCCCGACCAGCCCCAAGGTCTTCCCGCTGAGCCTCTGCAGCACCCAGCCAGATGGGAACGTGGTCATCGCCTGCCTGGTCCAGGGCTTCTTCCCCCAGGAGCCACTCAGTGTGACCTGGAGCGAAAGCGGACAGGGCGTGACCGCCAGAAACTTCCCACCCAGCCAGGATGCCTCCGGGGACCTGTACACCACGAGCAGCCAGCTGACCCTGCCGGCCACACAGTGCCTAGCCGGCAAGTCCGTGACATGCCACGTGAAGCACTACACGAATCCCAGCCAGGATGTGACTGTGCCCTGCCCAGTTCCCTCAACTCCACCTACCCCATCTCCCTCAACTCCACCTACCCCATCTCCCTCATGCTGCCACCCCCGACTGTCACTGCACCGACCGGCCCTCGAGGACCTGCTCTTAGGTTCAGAAGCGAACCTCACGTGCACACTGACCGGCCTGAGAGATGCCTCAGGTGTCACCTTCACCTGGACGCCCTCAAGTGGGAAGAGCGCTGTTCAAGGACCACCTGAGCGTGACCTCTGTGGCTGCTACAGCGTGTCCAGTGTCCTGCCGGGCTGTGCCGAGCCATGGAACCATGGGAAGACCTTCACTTGCACTGCTGCCTACCCCGAGTCCAAGACCCCGCTAACCGCCACCCTCTCAAAATCCGGAAACACATTCCGGCCCGAGGTCCACCTGCTGCCGCCGCCGTCGGAGGAGCTGGCCCTGAACGAGCTGGTGACGCTGACGTGCCTGGCACGTGGCTTCAGCCCCAAGGATGTGCTGGTTCGCTGGCTGCAGGGGTCACAGGAGCTGCCCCGCGAGAAGTACCTGACTTGGGCATCCCGGCAGGAGCCCAGCCAGGGCACCACCACCTTCGCTGTGACCAGCATACTGCGCGTGGCAGCCGAGGACTGGAAGAAGGGGGACACCTTCTCCTGCATGGTGGGCCACGAGGCCCTGCCGCTGGCCTTCACACAGAAGACCATCGACCGCTTGGCGGGTAAACCCACCCATGTCAATGTGTCTGTTGTCATGGCGGAGGTGGACGGCACCTGCTACTGA

SEQ ID NO: 20 - protein, 318 aa, Homo sapiens
GTGGCTGCACCATCTGTCTTCATCTTCCCGCCATCTGATGAGCAGTTGAAATCTGGAACTGCCTCTGTTGTGTGCCTGCTGAATAACTTCTATCCCAGAGAGGCCAAAGTACAGTGGAAGGTGGATAACGCCCTCCAATCGGGTAACTCCCAGGAGAGTGTCACAGAGCAGGACAGCAAGGACAGCACCTACAGCCTCAGCAGCACCCTGACGCTGAGCAAAGCAGACTACGAGAAACACAAAGTCTACGCCTGCGAAGTCACCCATCAGGGCCTGAGCTCGCCCGTCACAAAGAGCTTCAACAGGGGAGAGTGTTAA